European Patent Application EP 4 299 072 A2, published January 3, 2024. Title: NOVEL ANTI-LAM AND ANTI-PIM6 MONOCLONAL ANTIBODIES FOR DIAGNOSIS AND TREATMENT OF MYCOBACTERIUM TUBERCULOSIS INFECTIONS. Applicant: Rutgers, The State University of New Jersey. Application EP. The sequence listing filed with the application follows.

SEQUENCE LISTING (50 sequences)

SEQ ID NO: 1 - protein, 6 aa, Homo sapiens
RSIRSA

SEQ ID NO: 2 - skipped

SEQ ID NO: 3 - protein, 9 aa, Homo sapiens
QQYDFWYTF

SEQ ID NO: 4 - protein, 8 aa, Homo sapiens
GFNFEDFG

SEQ ID NO: 5 - protein, 8 aa, Homo sapiens
ISWNGANI

SEQ ID NO: 6 - protein, 13 aa, Homo sapiens
IDWYRDDYYKMDV

SEQ ID NO: 7 - protein, 6 aa, Homo sapiens
QSINSN

SEQ ID NO: 8 - skipped

SEQ ID NO: 9 - protein, 9 aa, Homo sapiens
QQYKAFKTF

SEQ ID NO: 10 - protein, 8 aa, Homo sapiens
GGSFSGYY

SEQ ID NO: 11 - protein, 13 aa, Homo sapiens
FDLGGSITHSRGT

SEQ ID NO: 12 - protein, 13 aa, Homo sapiens
RGLAMGGTKEFDS

SEQ ID NO: 13 - protein, 12 aa, Homo sapiens
QNVLDSANNRNY

SEQ ID NO: 14 - skipped

SEQ ID NO: 15 - protein, 9 aa, Homo sapiens
TQYHRLPHT

SEQ ID NO: 16 - protein, 9 aa, Homo sapiens
GGSINTNNW

SEQ ID NO: 17 - protein, 7 aa, Homo sapiens
IHRHGDT

SEQ ID NO: 18 - protein, 15 aa, Homo sapiens
CPLGYCSGDDCHRVA

SEQ ID NO: 19 - protein, 5 aa, Homo sapiens
GGSGG

SEQ ID NO: 20 - skipped

SEQ ID NO: 21 - protein, 96 aa, Homo sapiens
QVQLLESGGGVVRPGGSLRLSCAASGFNFEDFGMSWVRQAPGKGLEWVSSISWNGANIGYVDSVKGRFTISRDNAKNSLYLQMNSLRAEDTALYYC

SEQ ID NO: 22 - protein, 96 aa, Homo sapiens
EVQLVESGGGVVRPGGSLRLSCAASGFTFDDYGMSWVRQAPGKGLEWVSGINWNGGSTGYADSVKGRFTISRDNAKNSLYLQMNSLRAEDTALYHC

SEQ ID NO: 23 - protein, 14 aa, Homo sapiens
AIDWYRDDYYKMDV

SEQ ID NO: 24 - protein, 88 aa, Homo sapiens
EIVMTQSPATLSVSPGERATLSCRASRSIRSALAWYQHKPGQAPRLLIFGASTRATGIPARFSGSGSGTDFTLTVSSIRSEDSAVYYC

SEQ ID NO: 25 - protein, 88 aa, Homo sapiens
EIVMTQSPATLSVSPGERATLSCRASQSVSSNLAWYQQKPGQAPRLLIYGASTRATGIPARFSGSGSGTEFTLTISSLQSEDFAVYYC

SEQ ID NO: 26 - protein, 8 aa, Homo sapiens
QQYDFWYT

SEQ ID NO: 27 - protein, 101 aa, Homo sapiens
QVQLQQWGAGLLKPSETLSLTCAVYGGSFSGYYWSWIRQSPETGLEWLGEFDLGGSITHSRGTNYNPSLKSRVTISGDTSKNQFSLKLTSVTAADTAVYYC

SEQ ID NO: 28 - protein, 95 aa, Homo sapiens
QVQLQQWGAGLLKPSETLSLTCAVYGGSFSGYYWSWIRQPPGKGLEWIGEINHSGSTNYNPSLKSRVTISVDTSKNQFSLKLSSVTAADTAVYYC

SEQ ID NO: 29 - protein, 14 aa, Homo sapiens
ARGLAMGGTKEFDS

SEQ ID NO: 30 - protein, 88 aa, Homo sapiens
DIQMTQSPDSLSASVGDRITITCRASQSINSNLAWYQQKPGKAPKLLIYKASDLESGVPSRFSGSGSGTEFTLTISSLQPDDFATYYC

SEQ ID NO: 31 - protein, 88 aa, Homo sapiens
DIQMTQSPSTLSASVGDRVTITCRASQSISSWLAWYQQKPGKAPKLLIYKASSLESGVPSRFSGSGSGTEFTLTISSLQPDDFATYYC

SEQ ID NO: 32 - protein, 8 aa, Homo sapiens
QQYKAFKT

SEQ ID NO: 33 - protein, 96 aa, Homo sapiens
EVQLLESGPGLVRPWGTLSLTCAVSGGSINTNNWWSWVRQSPGKGLEWIGEIHRHGDTNYNPSLKRRVSISMDESMNQFSLRLISVTAADTAVYYC

SEQ ID NO: 34 - protein, 96 aa, Homo sapiens
QVQLQESGPGLVKPSGTLSLTCAVSGGSISSSNWWSWVRQPPGKGLEWIGEIYHSGSTNYNPSLKSRVTISVDKSKNQFSLKLSSVTAADTAVYYC

SEQ ID NO: 35 - skipped

SEQ ID NO: 36 - protein, 94 aa, Homo sapiens
DIQMTQSPSSLSVSLGERATINCKSSQNVLDSANNRNYFGWYQQKPGQPPKLLISWASTRESGVPDRFSGSGSGTDFTLIISGLQVEDVAVYYC

SEQ ID NO: 37 - protein, 94 aa, Homo sapiens
DIVMTQSPDSLAVSLGERATINCKSSQSVLYSSNNKNYLAWYQQKPGQPPKLLIYWASTRESGVPDRFSGSGSGTDFTLTISSLQAEDVAVYYC

SEQ ID NO: 38 - skipped

SEQ ID NO: 39 - DNA, 1356 bp, Homo sapiens
  source 1..1356: mol_type = unassigned DNA
caagtgcagctgttggagtctgggggaggtgtggtacggccgggggggtccctgagactctcctgtgcagcctctggattcaactttgaagattttggcatgagctgggtccgccaagctccagggaaggggctggagtgggtctctagtattagttggaatggtgctaatataggctatgtagactctgtgaagggccgattcaccatctccagagacaacgccaagaactccctatatctgcaaatgaacagtctgagagccgaggacacggccttatattactgtgcgatagactggtacagagacgactactacaagatggacgtctggggcaaagggaccacggtcaccgtctcctcagcctcgaccaagggcccatcggtcttcccgctagcgccctcctccaagagcacctctgggggcacagcggccctgggctgcctggtcaaggactacttccccgaacctgtgacggtctcgtggaactcaggcgccctgaccagcggcgtgcacaccttcccggctgtcctacagtcctcaggactctactccctcagcagcgtggtgaccgtgccctccagcagcttgggcacccagacctacatctgcaacgtgaatcacaagcccagcaacaccaaggtggacaagaaagttgagcccaaatcttgtgacaaaactcacacatgcccaccgtgcccagcacctgaactcctggggggaccgtcagtcttcctcttccccccaaaacccaaggacaccctcatgatctcccggacccctgaggtcacatgcgtggtggtggacgtgagccacgaagaccctgaggtcaagttcaactggtacgtggacggcgtggaggtgcataatgccaagacaaagccgcgggaggagcagtacaacagcacgtaccgtgtggtcagcgtcctcaccgtcctgcaccaggactggctgaatggcaaggagtacaagtgcaaggtctccaacaaagccctcccagcccccatcgagaaaaccatctccaaagccaaagggcagccccgagaaccacaggtgtacaccctgcccccatcccgggatgagctgaccaagaaccaggtcagcctgacctgcctggtcaaaggcttctatcccagcgacatcgccgtggagtgggagagcaatgggcagccggagaacaactacaagaccacgcctcccgtgctggactccgacggctccttcttcctctacagcaagctcaccgtggacaagagcaggtggcagcaggggaacgtcttctcatgctccgtgatgcatgaggctctgcacaaccactacacgcagaagagcctctccctgtctccgggtaaatga

SEQ ID NO: 40 - protein, 451 aa, Homo sapiens
QVQLLESGGGVVRPGGSLRLSCAASGFNFEDFGMSWVRQAPGKGLEWVSSISWNGANIGYVDSVKGRFTISRDNAKNSLYLQMNSLRAEDTALYYCAIDWYRDDYYKMDVWGKGTTVTVSSASTKGPSVFPLAPSSKSTSGGTAALGCLVKDYFPEPVTVSWNSGALTSGVHTFPAVLQSSGLYSLSSVVTVPSSSLGTQTYICNVNHKPSNTKVDKKVEPKSCDKTHTCPPCPAPELLGGPSVFLFPPKPKDTLMISRTPEVTCVVVDVSHEDPEVKFNWYVDGVEVHNAKTKPREEQYNSTYRVVSVLTVLHQDWLNGKEYKCKVSNKALPAPIEKTISKAKGQPREPQVYTLPPSRDELTKNQVSLTCLVKGFYPSDIAVEWESNGQPENNYKTTPPVLDSDGSFFLYSKLTVDKSRWQQGNVFSCSVMHEALHNHYTQKSLSLSPGK

SEQ ID NO: 41 - DNA, 642 bp, Homo sapiens
  source 1..642: mol_type = unassigned DNA
gaaatagtgatgacgcagtctccagccaccctgtctgtctctccaggggaaagagccaccctctcctgcagggccagtcggagtattcgcagcgccttagcctggtaccagcacaaacctggccaggctcccaggctcctcatctttggtgcatccaccagggccactggtatcccagccaggttcagtggcagtgggtctgggacagacttcactctcaccgtcagcagcatacggtctgaggattctgcagtttattactgtcagcagtatgatttctggtacacttttggccaggggaccaagctggagatcaaacgaactgtggctgcaccatctgtcttcatcttcccgccatctgatgagcagttgaaatctggaactgcctctgttgtgtgcctgctgaataacttctatcccagagaggccaaagtacagtggaaggtcgacaacgccctccaatcgggtaactcccaggagagtgtcacagagcaggacagcaaggacagcacctacagcctcagcagcaccctgacgctgagcaaagcagactacgagaaacacaaagtctacgcctgcgaagtcacccatcagggcctgagctcgcccgtcacaaagagcttcaacaggggagagtgttag

SEQ ID NO: 42 - protein, 213 aa, Homo sapiens
EIVMTQSPATLSVSPGERATLSCRASRSIRSALAWYQHKPGQAPRLLIFGASTRATGIPARFSGSGSGTDFTLTVSSIRSEDSAVYYCQQYDFWYTFGQGTKLEIKRTVAAPSVFIFPPSDEQLKSGTASVVCLLNNFYPREAKVQWKVDNALQSGNSQESVTEQDSKDSTYSLSSTLTLSKADYEKHKVYACEVTHQGLSSPVTKSFNRGEC

SEQ ID NO: 43 - protein, 115 aa, Homo sapiens
QVQLQQWGAGLLKPSETLSLTCAVYGGSFSGYYWSWIRQSPETGLEWLGEFDLGGSITHSRGTNYNPSLKSRVTISGDTSKNQFSLKLTSVTAADTAVYYCARGLAMGGTKEFDS

SEQ ID NO: 44 - protein, 96 aa, Homo sapiens
DIQMTQSPDSLSASVGDRITITCRASQSINSNLAWYQQKPGKAPKLLIYKASDLESGVPSRFSGSGSGTEFTLTISSLQPDDFATYYCQQYKAFKT

SEQ ID NO: 45 - DNA, 379 bp, Homo sapiens
  source 1..379: mol_type = unassigned DNA
caggtgcagctacagcagtggggcgcaggactgttgaagccttcggagaccctgtccctcacctgcgctgtctatggtgggtccttcagtggttactactggagctggatccgccagtccccagagacggggctggagtggcttggcgaattcgatcttggtggaagcatcactcatagtagaggcaccaactacaacccgtcgctcaagagtcgagtcaccatctcaggagacacgtccaagaaccagttctccctgaaactgacctctgtgaccgccgcggacacggctgtctattactgtgcgagaggtttagcaatgggtggaactaaggagtttgactcctggggccagggaaccctggtcaccgtctcctcag

SEQ ID NO: 46 - DNA, 319 bp, Homo sapiens
  source 1..319: mol_type = unassigned DNA
gacatccagatgacccagtctccagactccctgtctgcatctgtaggagacagaatcaccatcacttgccgggccagtcagagtattaatagtaatttggcctggtatcagcagaaaccggggaaagcccctaagctcctgatctataaggcgtctgatttagaaagtggggtcccatcaaggttcagcggcagtggatctgggacagaattcactctcaccatcagcagcctgcagcctgatgattttgcaacttattattgccaacagtataaagcattcaagacgttcggccacgggaccaaggtggaaatcaaac

SEQ ID NO: 47 - protein, 111 aa, Homo sapiens
EVQLLESGPGLVRPWGTLSLTCAVSGGSINTNNWWSWVRQSPGKGLEWIGEIHRHGDTNYNPSLKRRVSISMDESMNQFSLRLISVTAADTAVYYCCPLGYCSGDDCHRVA

SEQ ID NO: 48 - protein, 103 aa, Homo sapiens
DIQMTQSPSSLSVSLGERATINCKSSQNVLDSANNRNYFGWYQQKPGQPPKLLISWASTRESGVPDRFSGSGSGTDFTLIISGLQVEDVAVYYCTQYHRLPHT

SEQ ID NO: 49 - DNA, 367 bp, Homo sapiens
  source 1..367: mol_type = unassigned DNA
gaggtgcagctcttggagtcgggcccaggactggtgaggccttgggggactctgtccctcacctgcgctgtctctggtggctccatcaatactaataactggtggagttgggtccgccagtccccggggaaggggctggagtggattggagaaatccatcgtcatggggacaccaactacaacccgtcactcaagaggcgagtctccatatcgatggacgagtccatgaaccagttctccctgaggcttatctctgtgaccgccgcggacacggccgtgtattactgttgtcccctaggatattgtagtggtgatgactgtcaccgagttgcctggggccggggaatcctggtcaccgtctcttcag

SEQ ID NO: 50 - DNA, 340 bp, Homo sapiens
  source 1..340: mol_type = unassigned DNA
gacatccagatgacccagtctccatcctccctgtctgtgtctctgggcgagagggccaccatcaactgcaagtccagccagaatgttttagacagcgccaacaataggaactacttcggttggtaccagcagaaaccagggcagcctcctaagctgctcatttcctgggcatctacacgggaatccggggtccctgaccgattcagtggcagcggctctgggacagacttcactctcatcatcagcggcctgcaggttgaagatgtggcagtttattactgtacacagtatcatagacttcctcacaccttcggccaagggacacgactggaaattaaac